European Patent Application EP 4 686 755 A1, published February 4, 2026. Title: Proteinaceous nanocapsules with oxide-dependent open-close capability. Applicant: Uniwersytet Jagiellonski. Application EP. The sequence listing filed with the application follows.

SEQUENCE LISTING (71 sequences)

SEQ ID NO: 1 - protein, 154 aa, Aquifex aeolicus
MEIYEGKLTAEGLRFGIVASRFNHALVDRLVEGAIHCIVRHGGREEDITLVRVPGSWEIPVAAGELARKEDIDAVIAIGVLIRGATPHFDYIASEVSKGLANLSLELRKPITFGVITADTIEQALERAGTKHGNKGWEAALSAIEMANLFKSLR

SEQ ID NO: 2 - protein, 154 aa, synthetic construct
MEIYEGKLTAEGLRFGIVASXFNHALVDRLVXGAIHCIVRHGGREEDITLVRVPGSWEIPVAAGELARKEDIDAVIAIGVLIRGATPHFDYIASEVSKGLANLSLELRKPITFGVITADTXEQAXERAGTKHGNKGWEAALSAIEMANLFKSLR

SEQ ID NO: 3 - protein, 154 aa, synthetic construct
MEIYEGKLTAEGLRFGIVASXFNHALVDRLVXGAIHCIVXXGGREEDITLVRVPGSWEIPVAAGELARKEDIDAVIAIGVLIRGATPHFDYIASEVSKGLANLSLELRKPITFGVITADTXEQAXERAGTKHGNKGWEAALSAIEMANLFKSLR

SEQ ID NO: 4 - protein, 156 aa, synthetic construct
MATPHFDYIASEVSKGLANLSLELRKPITFGVITADTLEQAIERAGTKHGNKGWEAALSAIEMANLFKSLRXMEIYEGKLTAEGLRFGIVASRFNHALVDRLVEGAIDCIVRHGGREEDITLVRVPGSWEIPVAAGELARKEDIDAVIAIGVLIRG

SEQ ID NO: 5 - protein, 156 aa, synthetic construct
MTLEQAIERAGTKHGNKGWEAALSAIEMANLFKSLRXMEIYEGKLTAEGLRFGIVASRFNHALVDRLVEGAIDCIVRHGGREEDITLVRVPGSWEIPVAAGELARKEDIDAVIAIGVLIRGATPHFDYIASEVSKGLANLSLELRKPITFGVITAD

SEQ ID NO: 6 - protein, 154 aa, synthetic construct
MEIYEGKLTAEGLRFGIVASCFNHALVDRLVHGAIHCIVRHGGREEDITLVRVPGSWEIPVAAGELARKEDIDAVIAIGVLIRGATPHFDYIASEVSKGLANLSLELRKPITFGVITADTLEQAHERAGTKHGNKGWEAALSAIEMANLFKSLR

SEQ ID NO: 7 - protein, 154 aa, synthetic construct
MEIYEGKLTAEGLRFGIVASCFNHALVDRLVHGAIHCIVRHGGREEDITLVRVPGSWEIPVAAGELARKEDIDAVIAIGVLIRGATPHFDYIASEVSKGLANLSLELRKPITFGVITADTLEQASERAGTKHGNKGWEAALSAIEMANLFKSLR

SEQ ID NO: 8 - protein, 154 aa, synthetic construct
MEIYEGKLTAEGLRFGIVASCFNHALVDRLVHGAISCIVRHGGREEDITLVRVPGSWEIPVAAGELARKEDIDAVIAIGVLIRGATPHFDYIASEVSKGLANLSLELRKPITFGVITADTLEQAHERAGTKHGNKGWEAALSAIEMANLFKSLR

SEQ ID NO: 9 - protein, 154 aa, synthetic construct
MEIYEGKLTAEGLRFGIVASCFNHALVDRLVSGAIDCIVRHGGREEDITLVRVPGSWEIPVAAGELARKEDIDAVIAIGVLIRGATPHFDYIASEVSKGLANLSLELRKPITFGVITADTLEQAHERAGTKHGNKGWEAALSAIEMANLFKSLR

SEQ ID NO: 10 - protein, 154 aa, synthetic construct
MEIYEGKLTAEGLRFGIVASCFNHALVDRLVSGAIHCIVRHGGREEDITLVRVPGSWEIPVAAGELARKEDIDAVIAIGVLIRGATPHFDYIASEVSKGLANLSLELRKPITFGVITADTLEQAHERAGTKHGNKGWEAALSAIEMANLFKSLR

SEQ ID NO: 11 - protein, 154 aa, synthetic construct
MEIYEGKLTAEGLRFGIVASCFNHALVDRLVHGAIHCIVRHGGREEDITLVRVPGSWEIPVAAGELARKEDIDAVIAIGVLIRGATPHFDYIASEVSKGLANLSLELRKPITFGVITADTSEQAIERAGTKHGNKGWEAALSAIEMANLFKSLR

SEQ ID NO: 12 - protein, 154 aa, synthetic construct
MEIYEGKLTAEGLRFGIVASCFNHALVDRLVHGAIHCIVRHGGREEDITLVRVPGSWEIPVAAGELARKEDIDAVIAIGVLIRGATPHFDYIASEVSKGLANLSLELRKPITFGVITADTLEQAAERAGTKHGNKGWEAALSAIEMANLFKSLR

SEQ ID NO: 13 - protein, 154 aa, synthetic construct
MEIYEGKLTAEGLRFGIVASCFNHALVDRLVHGAIHCIVSHGGREEDITLVRVPGSWEIPVAAGELARKEDIDAVIAIGVLIRGATPHFDYIASEVSKGLANLSLELRKPITFGVITADTLEQAHERAGTKHGNKGWEAALSAIEMANLFKSLR

SEQ ID NO: 14 - protein, 154 aa, synthetic construct
MEIYEGKLTAEGLRFGIVASCFNHALVDRLVHGAIHCIVRSGGREEDITLVRVPGSWEIPVAAGELARKEDIDAVIAIGVLIRGATPHFDYIASEVSKGLANLSLELRKPITFGVITADTLEQAHERAGTKHGNKGWEAALSAIEMANLFKSLR

SEQ ID NO: 15-22 - skipped (8 entries)

SEQ ID NO: 23 - protein, 154 aa, synthetic construct
MEIYEGKLTAEGLRFGIVASCFNHALVDALVHGAIHCIVRHGGREEDITLVRVPGSWEIPVAAGELARKEDIDAVIAIGVLIRGATPHFDYIASEVSKGLANLSLELRKPITFGVITADTLEQAHERAGTKHGNKGWEAALSAIEMANLFKSLR

SEQ ID NO: 24-26 - skipped (3 entries)

SEQ ID NO: 27 - protein, 432 aa, synthetic construct
MTLEQAIERAGTKHGNKGWEAALSAIEMANLFKSLRGTGGSGSSMEIYEGKLTAEGLRFGIVASRFNHALVDRLVEGAIDCIVRHGGREEDITLVRVPGSWEIPVAAGELARKEDIDAVIAIGVLIRGATPHFDYIASEVSKGLANLSLELRKPITFGVITADAGGAGGSENLYFQSGGSGSKGEELFTGVVPILVELDGDVNGHKFSVRGEGEGDATNGKLTLKFICTTGKLPVPWPTLVTTLTYGVQCFSRYPDHMKRHDFFKSAMPEGYVQERTISFKDDGTYKTRAEVKFEGDTLVNRIELKGIDFKEDGNILGHKLEYNFNSHNVYITADKQKNGIKANFKIRHNVEDGSVQLADHYQQNTPIGDGPVLLPDNHYLSTQSKLSKDPNEKRDHMVLLEFVTAAGITHGMDELYKTNSAANDENYALAA

SEQ ID NO: 28-69 - skipped (42 entries)

SEQ ID NO: 70 - protein, 8 aa, synthetic construct
GTGGSGSS

SEQ ID NO: 71 - protein, 12 aa, synthetic construct
LEGGWSHPQFEK